European Patent Application EP 4 151 653 A1, published March 22, 2023. Title: CD22-TARGETED CHIMERIC ANTIGEN RECEPTOR, PREPARATION METHOD THEREFOR AND APPLICATION THEREOF. Applicant: SHANGHAI CELLULAR BIOPHARMACEUTICAL GROUP LTD. WUXI CELLULAR BIOPHARMACEUTICAL GROUP LTD. The sequence listing filed with the application follows.

SEQUENCE LISTING (16 sequences)

SEQ ID NO: 1 - protein, 121 aa, Artificial Sequence
  Heavy chain variable domain
EVQLVQSGAEVKKPGESLKISCKGSGYNFTSYWIGWVRQMPGKGLEWMGIIYPGDSDTRYSPSFQGQVTISADKSISTAYLQWSSLKASDTAMYYCATPTYYFGSVAFDIWGQGTMVTVSS

SEQ ID NO: 2 - protein, 107 aa, Artificial Sequence
  Light chain variable domain
EIVLTQSPDFQSVTPKEKVTITCRASQSIGSSLHWYQQKPDQSPKLLIKYASQSFSGVPSRFSGSGSGTDFTLTINSLEAEDAAAYYCHQSSSLPYTFGQGTKLEIK

SEQ ID NO: 3 - protein, 122 aa, Artificial Sequence
  Heavy chain variable domain
QVQLVQSGAEVKKPGSSVKVSCKPSGDTFSNYAISWVRQAPGQGLEWMGRIIPILGMAIYAPKFQGRVTITADKSTNTAFMDLTSLYFEDTAVYYCARAPTYWGSKDYFDYWGQGTLVTVSS

SEQ ID NO: 4 - protein, 107 aa, Artificial Sequence
  Light chain variable domain
AIQLTQSPSSLSASVGDRVTITCRASQDISSGLAWYQQKPGTAPKLLIYDASSLESGVPSRFSGSGSGTDFTLTISSLQPDDFATYYCQQFNSFPYTFGQGTKLEIK

SEQ ID NO: 5 - protein, 123 aa, Artificial Sequence
  Heavy chain variable domain
EVQLVESGGGLVQPGGSLRLSCAASGFAFSIYDMSWVRQVPGKGLEWVSYISSGGGTTYYPDTVKGRFTISRDNSRNTLDLQMNSLRVEDTAVYYCARHSGYGSSYGVLFAYWGQGTLVTVSS

SEQ ID NO: 6 - protein, 107 aa, Artificial Sequence
  Light chain variable domain
DIQMTQSPSSLSASVGDRVTITCRASQDISNYLNWLQQKPGKAPKLLIYYTSILHSGVPSRFSGSGSGTEFTLTISSLQPEDFATYYCQQGNTLPWTFGQGTKLEIK

SEQ ID NO: 7 - protein, 120 aa, Artificial Sequence
  Heavy chain variable domain
LQQSGPGLVKPSQTLSLTCAISGDSVSSNSAAWNWIRQSPSRGLEWLGRTYYRSKWYNDYAVSVKSRITINPDTSKNQFSLQLNSVTPEDTAVYYCAREVTGDLEDAFDIWGQGTMVTVS

SEQ ID NO: 8 - protein, 105 aa, Artificial Sequence
  Light chain variable domain
IQMTQSPSSLSASVGDRVTITCRASQTIWSYLNWYQQRPGKAPNLLIYAASSLQSGVPSRFSGRGSGTDFTLTISSLQAEDFATYYCQQSYSIPQTFGQGTKLEI

SEQ ID NO: 9 - protein, 21 aa, Artificial Sequence
  Signal peptide
MALPVTALLLPLALLLHAARP

SEQ ID NO: 10 - protein, 55 aa, Artificial Sequence
  Hinge region
FVPVFLPAKPTTTPAPRPPTPAPTIASQPLSLRPEACRPAAGGAVHTRGLDFACD

SEQ ID NO: 11 - protein, 24 aa, Artificial Sequence
  Transmembrane region
IYIWAPLAGTCGVLLLSLVITLYC

SEQ ID NO: 12 - protein, 42 aa, Artificial Sequence
  Co-stimulatory signaling molecule
KRGRKKLLYIFKQPFMRPVQTTQEEDGCSCRFPEEEEGGCEL

SEQ ID NO: 13 - protein, 113 aa, Artificial Sequence
  CD3? signaling sequence
RVKFSRSADAPAYQQGQNQLYNELNLGRREEYDVLDKRRGRDPEMGGKPQRRKNPQEGLYNELQKDKMAEAYSEIGMKGERRRGKGHDGLYQGLSTATKDTYDALHMQALPPR

SEQ ID NO: 14 - protein, 497 aa, Artificial Sequence
  Chimeric antigen receptor
MALPVTALLLPLALLLHAARPEVQLVQSGAEVKKPGESLKISCKGSGYNFTSYWIGWVRQMPGKGLEWMGIIYPGDSDTRYSPSFQGQVTISADKSISTAYLQWSSLKASDTAMYYCATPTYYFGSVAFDIWGQGTMVTVSSGGGGSGGGGSGGGGSEIVLTQSPDFQSVTPKEKVTITCRASQSIGSSLHWYQQKPDQSPKLLIKYASQSFSGVPSRFSGSGSGTDFTLTINSLEAEDAAAYYCHQSSSLPYTFGQGTKLEIKFVPVFLPAKPTTTPAPRPPTPAPTIASQPLSLRPEACRPAAGGAVHTRGLDFACDIYIWAPLAGTCGVLLLSLVITLYCKRGRKKLLYIFKQPFMRPVQTTQEEDGCSCRFPEEEEGGCELRVKFSRSADAPAYQQGQNQLYNELNLGRREEYDVLDKRRGRDPEMGGKPRRKNPQEGLYNELQKDKMAEAYSEIGMKGERRRGKGHDGLYQGLSTATKDTYDALHMQALPPR

SEQ ID NO: 15 - protein, 498 aa, Artificial Sequence
  Chimeric antigen receptor
MALPVTALLLPLALLLHAARPQVQLVQSGAEVKKPGSSVKVSCKPSGDTFSNYAISWVRQAPGQGLEWMGRIIPILGMAIYAPKFQGRVTITADKSTNTAFMDLTSLYFEDTAVYYCARAPTYWGSKDYFDYWGQGTLVTVSSGGGGSGGGGSGGGGSAIQLTQSPSSLSASVGDRVTITCRASQDISSGLAWYQQKPGTAPKLLIYDASSLESGVPSRFSGSGSGTDFTLTISSLQPDDFATYYCQQFNSFPYTFGQGTKLEIKFVPVFLPAKPTTTPAPRPPTPAPTIASQPLSLRPEACRPAAGGAVHTRGLDFACDIYIWAPLAGTCGVLLLSLVITLYCKRGRKKLLYIFKQPFMRPVQTTQEEDGCSCRFPEEEEGGCELRVKFSRSADAPAYQQGQNQLYNELNLGRREEYDVLDKRRGRDPEMGGKPRRKNPQEGLYNELQKDKMAEAYSEIGMKGERRRGKGHDGLYQGLSTATKDTYDALHMQALPPR

SEQ ID NO: 16 - protein, 15 aa, Artificial Sequence
  Linker peptide
GGGGSGGGGSGGGGS